European Patent Application EP 4 574 155 A1, published June 25, 2025. Title: Molecules for use in cell regeneration and rejuvenation. Applicant: Christine Süßmuth. Application EP. The sequence listing filed with the application follows.

SEQUENCE LISTING (7 sequences)

SEQ ID NO: 1 - DNA, 1920 bp, Homo sapiens
  source 1..1920: mol_type = other DNA
ctttttaagctcccctgagccggtgctgcgctcctctaattgggactccgagccggggctatttctggcgctggcgcggctccaagaaggcatccgcatttgctaccagcggcggccgcggcggagccaggccggtcctcagcgcccagcaccgccgctcccggcaacccggagcgcgcaccgcaggccggcggccgagctcgcgcatcccagccatcactcttccacctgctccttagagaagggaagatgagtgagtcgagctcgaagtccagccagcccttggcctccaagcaggaaaaggacggcactgagaagcggggccggggcaggccgcgcaagcagcctccggtgagtcccgggacagcgctggtagggagtcagaaggagcccagcgaagtgccaacacctaagagacctcggggccgaccaaagggaagcaaaaacaagggtgctgccaagacccggaaaaccaccacaactccaggaaggaaaccaaggggcagacccaaaaaactggagaaggaggaagaggagggcatctcgcaggagtcctcggaggaggagcagtgacccatgcgtgccgcctgctcctcactggaggagcagcttccttctgggactggacagctttgctccgctcccaccgcccccaccccttccccaggcccaccatcaccaccgcctctggccgccacccccatcttccacctgtgccctcaccaccacactacacagcacaccagccgctgcagggctcccatgggctgagtggggagcagttttcccctggcctcagttcccagctccccccgcccacccacgcatacacacatgccctcctggacaaggctaacatcccacttagccgcaccctgcacctgctgcgtccccactcccttggtggtggggacattgctctctgggcttttggtttgggggcgccctctctgctccttcactgttccctctggcttcccatagtggggcctgggagggttcccctggccttaaaaggggcccaagccccatctcatcctggcacgccctactccactgccctggcagcagcaggtgtggccaatggaggggggtgctggcccccaggattcccccagccaaactgtctttgtcaccacgtggggctcacttttcatccttccccaacttccctagtccccgtactaggttggacagcccccttcggttacaggaaggcaggaggggtgagtcccctactccctcttcactgtggccacagcccccttgccctccgcctgggatctgagtacatattgtggtgatggagatgcagtcacttattgtccaggtgaggcccaagagccctgtggccgccacctgaggtgggctggggctgctcccctaaccctactttgcttccgccactcagccatttccccctcctcagatggggcaccaataacaaggagctcaccctgcccgctcccaacccccctcctgctcctccctgccccccaaggttctggttccatttttcctctgttcacaaactacctctggacagttgtgttgttttttgttcaatgttccattcttcgacatccgtcattgctgctgctaccagcgccaaatgttcatcctcattgcctcctgttctgcccacgatcccctcccccaagatactctttgtggggaagaggggctggggcatggcaggctgggtgaccgactaccccagtcccagggaaggtggggccctgcccctaggatgctgcagcagagtgagcaagggggcccaaatcgaccataaagggtgtaggggccacctcctccccctgttctgttggggaggggtagccatgatttgtcccagcctggggctccctctctggtttcctatttgcagttacttgaataaaaaaaatatccttttctgga

SEQ ID NO: 2 - DNA, 324 bp, Homo sapiens
  source 1..324: mol_type = other DNA
atgagtgagtcgagctcgaagtccagccagcccttggcctccaagcaggaaaaggacggcactgagaagcggggccggggcaggccgcgcaagcagcctccggtgagtcccgggacagcgctggtagggagtcagaaggagcccagcgaagtgccaacacctaagagacctcggggccgaccaaagggaagcaaaaacaagggtgctgccaagacccggaaaaccaccacaactccaggaaggaaaccaaggggcagacccaaaaaactggagaaggaggaagaggagggcatctcgcaggagtcctcggaggaggagcagtga

SEQ ID NO: 3 - protein, 107 aa, Homo sapiens
MSESSSKSSQPLASKQEKDGTEKRGRGRPRKQPPVSPGTALVGSQKEPSEVPTPKRPRGRPKGSKNKGAAKTRKTTTTPGRKPRGRPKKLEKEEEEGISQESSEEEQ

SEQ ID NO: 4 - DNA, 4117 bp, Homo sapiens
  source 1..4117: mol_type = other DNA
agaaaacttccagcccgggcagcgcgcgcttggtgcaagactcaggagctagcagcccgtccccctccgactctccggtgccgccgctgcctgctcccgccaccctaggaggcgcggtgccacccactactctgtcctctgcctgtgctccgtgcccgaccctatcccggcggagtctccccatcctcctttgctttccgactgcccaaggcactttcaatctcaatctcttctctctctctctctctctctctctctctctctctctctctctctctctctctctcgcagggtggggggaagaggaggaggaattctttccccgcctaacatttcaagggacacaattcactccaagtctcttccctttccaagccgcttccgaagtgctcccggtgcccgcaactcctgatcccaacccgcgagaggagcctctgcgacctcaaagcctctcttccttctccctcgcttccctcctcctcttgctacctccacctccaccgccacctccacctccggcacccacccaccgccgccgccgccaccggcagcgcctcctcctctcctcctcctcctcccctcttctctttttggcagccgctggacgtccggtgttgatggtggcagcggcggcagcctaagcaacagcagccctcgcagcccgccagctcgcgctcgccccgccggcgtccccagccctatcacctcatctcccgaaaggtgctgggcagctccggggcggtcgaggcgaagcggctgcagcggcggtagcggcggcgggaggcaggatgagcgcacgcggtgagggcgcggggcagccgtccacttcagcccagggacaacctgccgccccagcgcctcagaagagaggacgcggccgccccaggaagcagcagcaagaaccaaccggtgagccctctcctaagagacccaggggaagacccaaaggcagcaaaaacaagagtccctctaaagcagctcaaaagaaagcagaagccactggagaaaaacggccaagaggcagacctaggaaatggccacaacaagttgttcagaagaagcctgctcaggaggaaactgaagagacatcctcacaagagtctgccgaagaggactagggggcgccaacgttcgatttctacctcagcagcagttggatcttttgaagggagaagacactgcagtgaccacttattctgtattgccatggtctttccactttcatctggggtggggtggggtggggtgggggaggggggggtggggtggggagaaatcacataaccttaaaaaggactatattaatcaccttctttgtaatcccttcacagtcccaggtttagtgaaaaactgctgtaaacacaggggacacagcttaacaatgcaacttttaattactgttttcttttttcttaacctactaatagtttgttgatctgataagcaagagtgggcgggtgagaaaaaccgaattgggtttagtcaatcactgcactgcatgcaaacaagaaacgtgtcacacttgtgacgtcgggcattcatataggaagaacgcggtgtgtaacactgtgtacacctcaaataccaccccaacccactccctgtagtgaatcctctgtttagaacaccaaagataaggactagatactactttctctttttcgtataatcttgtagacacttacttgatgatttttaactttttatttctaaatgagacgaaatgctgatgtatcctttcattcagctaacaaactagaaaaggttatgttcatttttcaaaaagggaagtaagcaaacaaatattgccaactcttctatttatggatatcacacatatcagcaggagtaataaatttactcacagcacttgttttcaggacaacacttcattttcaggaaatctacttcctacagagccaaaatgccatttagcaataaataacacttgtcagcctcagagcatttaaggaaactagacaagtaaaattatcctctttgtaatttaatgaaaaggtacaacagaataatgcatgatgaactcacctaattatgaggtgggaggagcgaaatctaaatttcttttgctatagttatacatcaatttaaaaagcaaaaaaaaaaaaggggggggcaatctctctctgtgtctttctctctctctcttcctctccctctctcttttcattgtgtatcagtttccatgaaagacctgaataccacttacctcaaattaagcatatgtgttacttcaagtaatacgttttgacataagatggttgaccaaggtgcttttcttcggcttgagttcaccatctcttcattcaaactgcacttttagccagagatgcaatatatccccactactcaatactacctctgaatgttacaacgaatttacagtctagtacttattacatgctgctatacacaagcaatgcaagaaaaaaacttactgggtaggtgattctaatcatctgcagttctttttgtacacttaattacagttaaagaagcaatctccttactgtgtttcagcatgactatgtatttttctatgtttttttaattaaaaatttttaaaatacttgtttcagcttctctgctagatttctacattaacttgaaaattttttaaccaagtcgctcctaggttcttaaggataattttcctcaatcacactacacatcacacaagatttgactgtaatatttaaatattaccctccaagtctgtacctcaaatgaattctttaaggagatggactaattgacttgcaaagacctacctccagacttcaaaaggaatgaacttgttacttgcagcattcatttgttttttcaatgtttgaaatagttcaaactgcagctaaccctagtcaaaactatttttgtaaaagacatttgatagaaaggaacacgtttttacatacttttgcaaaataagtaaataataaataaaataaaagccaaccttcaaagaaacttgaagctttgtaggtgagatgcaacaagccctgcttttgcataatgcaatcaaaaatatgtgtttttaagattagttgaatataagaaaatgcttgacaaatattttcatgtattttacacaaatgtgatttttgtaatatgtctcaaccagatttattttaaacgcttcttatgtagagtttttatgcctttctctcctagtgagtgtgctgactttttaacatggtattatcaactgggccaggaggtagtttctcatgacggcttttgtcagtatggcttttagtactgaagccaaatgaaactcaaaaccatctctcttccagctgcttcagggaggtagtttcaaaggccacatacctctctgagactggcagatcgctcactgttgtgaatcaccaaaggagctatggagagaattaaaactcaacattactgttaactgtgcgttaaataagcaaataaacagtggctcataaaaataaaagtcgcattccatatctttggatgggccttttagaaacctcattggccagctcataaaatggaagcaattgctcatgttggccaaacatggtgcaccgagtgatttccatctctggtaaagttacacttttatttcctgtatgttgtacaatcaaaacacactactacctcttaagtcccagtatacctcatttttcatactgaaaaaaaaagcttgtggccaatggaacagtaagaacatcataaaatttttatatatatagtttatttttgtgggagataaattttataggactgttctttgctgttgttggtcgcagctacataagactggacatttaacttttctaccatttctgcaagttaggtatgtttgcaggagaaaagtatcaagacgtttaactgcagttgactttctccctgttcctttgagtgtcttctaactttattctttgttctttatgtagaattgctgtctatgattgtactttgaatcgcttgcttgttgaaaatatttctctagtgtattatcactgtctgttctgcacaataaacataacagcctctgtgatccccatgtgttttgattcctgctctttgttacagttccattaaatgagtaataaagtttggtcaaaacaga

SEQ ID NO: 5 - DNA, 330 bp, Homo sapiens
  source 1..330: mol_type = other DNA
atgagcgcacgcggtgagggcgcggggcagccgtccacttcagcccagggacaacctgccgccccagcgcctcagaagagaggacgcggccgccccaggaagcagcagcaagaaccaaccggtgagccctctcctaagagacccaggggaagacccaaaggcagcaaaaacaagagtccctctaaagcagctcaaaagaaagcagaagccactggagaaaaacggccaagaggcagacctaggaaatggccacaacaagttgttcagaagaagcctgctcaggaggaaactgaagagacatcctcacaagagtctgccgaagaggactag

SEQ ID NO: 6 - protein, 109 aa, Homo sapiens
MSARGEGAGQPSTSAQGQPAAPAPQKRGRGRPRKQQQEPTGEPSPKRPRGRPKGSKNKSPSKAAQKKAEATGEKRPRGRPRKWPQQVVQKKPAQEETEETSSQESAEED

SEQ ID NO: 7 - DNA, 3009 bp, Homo sapiens
  source 1..3009: mol_type = genomic DNA
  misc_binding 21..28: bound_moiety = Let-7 binding seed site
  misc_binding 1107..1113: bound_moiety = Let-7 binding seed site
  misc_binding 1256..1262: bound_moiety = Let-7 binding seed site
  misc_binding 1619..1625: bound_moiety = Let-7 binding seed site
  misc_binding 1668..1674: bound_moiety = Let-7 binding seed site
  misc_binding 2521..2527: bound_moiety = Let-7 binding seed site
  misc_binding 2541..2547: bound_moiety = Let-7 binding seed site
ggggcgccaacgttcgatttctacctcagcagcagttggatcttttgaagggagaagacactgcagtgaccacttattctgtattgccatggtctttccactttcatctggggtggggtggggtggggtgggggaggggggggtggggtggggagaaatcacataaccttaaaaaggactatattaatcaccttctttgtaatcccttcacagtcccaggtttagtgaaaaactgctgtaaacacaggggacacagcttaacaatgcaacttttaattactgttttcttttttcttaacctactaatagtttgttgatctgataagcaagagtgggcgggtgagaaaaaccgaattgggtttagtcaatcactgcactgcatgcaaacaagaaacgtgtcacacttgtgacgtcgggcattcatataggaagaacgcggtgtgtaacactgtgtacacctcaaataccaccccaacccactccctgtagtgaatcctctgtttagaacaccaaagataaggactagatactactttctctttttcgtataatcttgtagacacttacttgatgatttttaactttttatttctaaatgagacgaaatgctgatgtatcctttcattcagctaacaaactagaaaaggttatgttcatttttcaaaaagggaagtaagcaaacaaatattgccaactcttctatttatggatatcacacatatcagcaggagtaataaatttactcacagcacttgttttcaggacaacacttcattttcaggaaatctacttcctacagagccaaaatgccatttagcaataaataacacttgtcagcctcagagcatttaaggaaactagacaagtaaaattatcctctttgtaatttaatgaaaaggtacaacagaataatgcatgatgaactcacctaattatgaggtgggaggagcgaaatctaaatttcttttgctatagttatacatcaatttaaaaagcaaaaaaaaaaaaggggggggcaatctctctctgtgtctttctctctctctcttcctctccctctctcttttcattgtgtatcagtttccatgaaagacctgaataccacttacctcaaattaagcatatgtgttacttcaagtaatacgttttgacataagatggttgaccaaggtgcttttcttcggcttgagttcaccatctcttcattcaaactgcacttttagccagagatgcaatatatccccactactcaatactacctctgaatgttacaacgaatttacagtctagtacttattacatgctgctatacacaagcaatgcaagaaaaaaacttactgggtaggtgattctaatcatctgcagttctttttgtacacttaattacagttaaagaagcaatctccttactgtgtttcagcatgactatgtatttttctatgtttttttaattaaaaatttttaaaatacttgtttcagcttctctgctagatttctacattaacttgaaaattttttaaccaagtcgctcctaggttcttaaggataattttcctcaatcacactacacatcacacaagatttgactgtaatatttaaatattaccctccaagtctgtacctcaaatgaattctttaaggagatggactaattgacttgcaaagacctacctccagacttcaaaaggaatgaacttgttacttgcagcattcatttgttttttcaatgtttgaaatagttcaaactgcagctaaccctagtcaaaactatttttgtaaaagacatttgatagaaaggaacacgtttttacatacttttgcaaaataagtaaataataaataaaataaaagccaaccttcaaagaaacttgaagctttgtaggtgagatgcaacaagccctgcttttgcataatgcaatcaaaaatatgtgtttttaagattagttgaatataagaaaatgcttgacaaatattttcatgtattttacacaaatgtgatttttgtaatatgtctcaaccagatttattttaaacgcttcttatgtagagtttttatgcctttctctcctagtgagtgtgctgactttttaacatggtattatcaactgggccaggaggtagtttctcatgacggcttttgtcagtatggcttttagtactgaagccaaatgaaactcaaaaccatctctcttccagctgcttcagggaggtagtttcaaaggccacatacctctctgagactggcagatcgctcactgttgtgaatcaccaaaggagctatggagagaattaaaactcaacattactgttaactgtgcgttaaataagcaaataaacagtggctcataaaaataaaagtcgcattccatatctttggatgggccttttagaaacctcattggccagctcataaaatggaagcaattgctcatgttggccaaacatggtgcaccgagtgatttccatctctggtaaagttacacttttatttcctgtatgttgtacaatcaaaacacactactacctcttaagtcccagtatacctcatttttcatactgaaaaaaaaagcttgtggccaatggaacagtaagaacatcataaaatttttatatatatagtttatttttgtgggagataaattttataggactgttctttgctgttgttggtcgcagctacataagactggacatttaacttttctaccatttctgcaagttaggtatgtttgcaggagaaaagtatcaagacgtttaactgcagttgactttctccctgttcctttgagtgtcttctaactttattctttgttctttatgtagaattgctgtctatgattgtactttgaatcgcttgcttgttgaaaatatttctctagtgtattatcactgtctgttctgcacaataaacataacagcctctgtgatccccatgtgttttgattcctgctctttgttacagttccattaaatgagtaataaagtttggtcaaaacagaaaaaaaaaaa